European Patent Specification EP 3 847 189 B1, published May 22, 2024. Title: UNIVERSAL DONOR CELLS. Applicant: CRISPR Therapeutics AG. The sequence listing filed with the application follows.

SEQUENCE LISTING (44 sequences)

SEQ ID NO: 1 - DNA, 20 bp, Homo sapiens
gctactctctctttctggcc

SEQ ID NO: 2 - DNA, 20 bp, Homo sapiens
ggccgagatgtctcgctccg

SEQ ID NO: 3 - DNA, 20 bp, Homo sapiens
cgcgagcacagctaaggcca

SEQ ID NO: 4 - DNA, 20 bp, Artificial Sequence
  Synthesized
cagacagcaaactcacccag

SEQ ID NO: 5 - DNA, 20 bp, Artificial Sequence
  Synthesized
aaactttgtcccgaccctcc

SEQ ID NO: 6 - DNA, 638 bp, Homo sapiens
cctagaatgagcgcccggtgtcccaagctggggcgcgcaccccagatcggcgggcgccgatgtacagacagcaaactcacccagtctagtgcatgccttcttaaacatcacgagactctagaaaaggaaactgaaaacgggaaagtccctctctctaacctggcactgcgtcgctggcttggagacaggtgacggtccctgcgggccttgtcctgattggctgggcacgcgtttaatataagtggaggcgtcgcgctggcgggcattcctgaagctgacagcattcgggccgagatgtctcgctccgtggccttagctgtgctcgcgctactctctctttctggcctggaggctatccagcgtgagtctctcctaccctcccgctctggtccttcctctcccgtctgcaccctctgtggccctcgctgtgctctctcgctccgtgacttcccttctccaagttctccttggtggcccgccgtggggctagtccagggctggatctcggggaagcggcggggtggcctgggagtggggaagggggtgcgcacccgggacgcgcgctacttgcccctttcggcggggagcaggggagacctttggcctacggcgacgggagggtcgggacaaagtttagg

SEQ ID NO: 7 - DNA, 20 bp, Artificial Sequence
  Synthesized
tctgcagaaggctaccccta

SEQ ID NO: 8 - DNA, 24 bp, Artificial Sequence
  Synthesized
tgctgtgtctaagacctctttcat

SEQ ID NO: 9 - DNA, 18 bp, Artificial Sequence
  Synthesized
gatttggacctgcgagcg

SEQ ID NO: 10 - DNA, 22 bp, Artificial Sequence
  Synthesized
caagcctggcaataaacaatga

SEQ ID NO: 11 - DNA, 15 bp, Artificial Sequence
  Synthesized
ctgctgcctgaacat

SEQ ID NO: 12 - DNA, 130 bp, Artificial Sequence
  Synthesized
cctgcaggcagctgcgcgctcgctcgctcactgaggccgcccgggcgtcgggcgacctttggtcgcccggcctcagtgagcgagcgagcgcgcagagagggagtggccaactccatcactaggggttcct

SEQ ID NO: 13 - DNA, 800 bp, Homo sapiens
gttctagggtggaaactaagagaatgatgtacctagagggcgctggaagctctaaagccctagcagttactgcttttactattagtggtcgtttttttctcccccccgccccccgacaaatcaacagaacaaagaaaattacctaaacagcaaggacatagggaggaacttcttggcacagaactttccaaacactttttcctgaagggatacaagaagcaagaaaggtactctttcactaggaccttctctgagctgtcctcaggatgcttttgggactatttttcttacccagagaatggagaaaccctgcagggaattcccaagctgtagttataaacagaagttctccttctgctaggtagcattcaaagatcttaatcttctgggtttccgttttctcgaatgaaaaatgcaggtccgagcagttaactggctggggcaccattagcaagtcacttagcatctctggggccagtctgcaaagcgagggggcagccttaatgtgcctccagcctgaagtcctagaatgagcgcccggtgtcccaagctggggcgcgcaccccagatcggagggcgccgatgtacagacagcaaactcacccagtctagtgcatgccttcttaaacatcacgagactctaagaaaaggaaactgaaaacgggaaagtccctctctctaacctggcactgcgtcgctggcttggagacaggtgacggtccctgcgggccttgtcctgattggctgggcacgcgtttaatataagtggaggcgtcgcgctggcgggcattcctgaagct

SEQ ID NO: 14 - DNA, 380 bp, Cytomegalovirus
gacattgattattgactagttattaatagtaatcaattacggggtcattagttcatagcccatatatggagttccgcgttacataacttacggtaaatggcccgcctggctgaccgcccaacgacccccgcccattgacgtcaataatgacgtatgttcccatagtaacgccaatagggactttccattgacgtcaatgggtggactatttacggtaaactgcccacttggcagtacatcaagtgtatcatatgccaagtacgccccctattgacgtcaatgacggtaaatggcccgcctggcattatgcccagtacatgaccttatgggactttcctacttggcagtacatctacgtattagtcatcgctattaccatg

SEQ ID NO: 15 - DNA, 276 bp, Gallus gallus
tcgaggtgagccccacgttctgcttcactctccccatctcccccccctccccacccccaattttgtatttatttattttttaattattttgtgcagcgatgggggcggggggggggggggcgcgcgccaggcggggcggggcggggcgaggggcggggcggggcgaggcggagaggtgcggcggcagccaatcagagcggcgcgctccgaaagtttccttttatggcgaggcggcggcggcggcggccctataaaaagcgaagcgcgcggcgggcg

SEQ ID NO: 16 - DNA, 1009 bp, Artificial Sequence
  Synthesized
ggagtcgctgcgttgccttcgccccgtgccccgctccgcgccgcctcgcgccgcccgccccggctctgactgaccgcgttactcccacaggtgagcgggcgggacggcccttctcctccgggctgtaattagcgcttggtttaatgacggctcgtttcttttctgtggctgcgtgaaagccttaaagggctccgggagggccctttgtgcgggggggagcggctcggggggtgcgtgcgtgtgtgtgtgcgtggggagcgccgcgtgcggcccgcgctgcccggcggctgtgagcgctgcgggcgcggcgcggggctttgtgcgctccgcgtgtgcgcgaggggagcgcggccgggggcggtgccccgcggtgcgggggggctgcgaggggaacaaaggctgcgtgcggggtgtgtgcgtgggggggtgagcagggggtgtgggcgcggcggtcgggctgtaacccccccctgcacccccctccccgagttgctgagcacggcccggcttcgggtgcggggctccgtgcggggcgtggcgcggggctcgccgtgccgggcggggggtggcggcaggtgggggtgccgggcggggcggggccgcctcgggccggggagggctcgggggaggggcgcggcggccccggagcgccggcggctgtcgaggcgcggcgagccgcagccattgccttttatggtaatcgtgcgagagggcgcagggacttcctttgtcccaaatctggcggagccgaaatctgggaggcgccgccgcaccccctctagcgggcgcgggcgaagcggtgcggcgccggcaggaaggaaatgggcggggagggccttcgtgcgtcgccgcgccgccgtccccttctccatctccagcctcggggctgccgcagggggacggctgccttcgggggggacggggcagggcggggttcggcttctggcgtgtgaccggcggctctagagcctctgctaaccatgttcatgccttcttctttttcctacag

SEQ ID NO: 17 - DNA, 873 bp, Homo sapiens
atgaggatatttgctgtctttatattcatgacctactggcatttgctgaacgcatttactgtcacggttcccaaggacctatatgtggtagagtatggtagcaatatgacaattgaatgcaaattcccagtagaaaaacaattagacctggctgcactaattgtctattgggaaatggaggataagaacattattcaatttgtgcatggagaggaagacctgaaggttcagcatagtagctacagacagagggcccggctgttgaaggaccagctctccctgggaaatgctgcacttcagatcacagatgtgaaattgcaggatgcaggggtgtaccgctgcatgatcagctatggtggtgccgactacaagcgaattactgtgaaagtcaatgccccatacaacaaaatcaaccaaagaattttggttgtggatccagtcacctctgaacatgaactgacatgtcaggctgagggctaccccaaggccgaagtcatctggacaagcagtgaccatcaagtcctgagtggtaagaccaccaccaccaattccaagagagaggagaaacttttcaatgtgaccagcacactgagaatcaacacaacaactaatgagattttctactgcacttttaggagattagatcctgaggaaaaccatacagctgaattggtcatcccagaactacctctggcacatcctccaaatgaaaggactcacttggtaattctgggagccatcttattatgccttggtgtagcactgacattcatcttccgtttaagaaaagggagaatgatggatgtgaaaaaatgtggcatccaagatacaaactcaaagaagcaaagtgatacacatttggaggagacgtaa

SEQ ID NO: 18 - DNA, 225 bp, Bos taurus
ctgtgccttctagttgccagccatctgttgtttgcccctcccccgtgccttccttgaccctggaaggtgccactcccactgtcctttcctaataaaatgaggaaattgcatcgcattgtctgagtaggtgtcattctattctggggggtggggtggggcaggacagcaagggggaggattgggaagacaatagcaggcatgctggggatgcggtgggctctatgg

SEQ ID NO: 19 - DNA, 800 bp, Homo sapiens
ccagcgtgagtctctcctaccctcccgctctggtccttcctctcccgctctgcaccctctgtggccctcgctgtgctctctcgctccgtgacttcccttctccaagttctccttggtggcccgccgtggggctagtccagggctggatctcggggaagcggcggggtggcctgggagtggggaagggggtgcgcacccgggacgcgcgctacttgcccctttcggcggggagcaggggagacctttggcctacggcgacgggagggtcgggacaaagtttagggcgtcgataagcgtcagagcgccgaggttgggggagggtttctcttccgctctttcgcggggcctctggctcccccagcgcagctggagtgggggacgggtaggctcgtcccaaaggcgcggcgctgaggtttgtgaacgcgtggaggggcgcttggggtctgggggaggcgtcgcccgggtaagcctgtctgctgcggctctgcttcccttagactggagagctgtggacttcgtctaggcgcccgctaagttcgcatgtcctagcacctctgggtctatgtggggccacaccgtggggaggaaacagcacgcgacgtttgtagaatgcttggctgtgatacaaagcggtttcgaataattaacttatttgttcccatcacatgtcacttttaaaaaattataagaactacccgttattgacatctttctgtgtgccaaggactttatgtgctttgcgtcatttaattttgaaaacagttatcttccgccatagataactactatggttatcttct

SEQ ID NO: 20 - DNA, 141 bp, Artificial Sequence
  Synthesized
aggaacccctagtgatggagttggccactccctctctgcgcgctcgctcgctcactgaggccgggcgaccaaaggtcgcccgacgcccgggctttgcccgggcggcctcagtgagcgagcgagcgcgcagctgcctgcagg

SEQ ID NO: 21 - DNA, 60 bp, Homo sapiens
atgtctcgctccgtggccttagctgtgctcgcgctactctctctttctggcctggaggct

SEQ ID NO: 22 - DNA, 27 bp, Homo sapiens
gtcatggcgccccgaaccctcttcctg

SEQ ID NO: 23 - DNA, 45 bp, Artificial Sequence
  Synthesized
ggtggaggcggttcaggcggaggtggctctggcggtggcggatcg

SEQ ID NO: 24 - DNA, 297 bp, Homo sapiens
atccagcgtactccaaagattcaggtttactcacgtcatccagcagagaatggaaagtcaaatttcctgaattgctatgtgtctgggtttcatccatccgacattgaagttgacttactgaagaatggagagagaattgaaaaagtggagcattcagacttgtctttcagcaaggactggtctttctatctcttgtactacactgaattcacccccactgaaaaagatgagtatgcctgccgtgtgaaccatgtgactttgtcacagcccaagatagttaagtgggatcgagacatg

SEQ ID NO: 25 - DNA, 60 bp, Artificial Sequence
  Synthesized
ggtggtggtggttctggtggtggtggttctggcggcggcggctccggtggtggtggatcc

SEQ ID NO: 26 - DNA, 1011 bp, Homo sapiens
ggctcccactccttgaagtatttccacacttccgtgtcccggcccggccgcggggagccccgcttcatctctgtgggctacgtggacgacacccagttcgtgcgcttcgacaacgacgccgcgagtccgaggatggtgccgcgggcgccgtggatggagcaggaggggtcagagtattgggaccgggagacacggagcgccagggacaccgcacagattttccgagtgaatctgcggacgctgcgcggctactacaatcagagcgaggccgggtctcacaccctgcagtggatgcatggctgcgagctggggcccgacgggcgcttcctccgcgggtatgaacagttcgcctacgacggcaaggattatctcaccctgaatgaggacctgcgctcctggaccgcggtggacacggcggctcagatctccgagcaaaagtcaaatgatgcctctgaggcggagcaccagagagcctacctggaagacacatgcgtggagtggctccacaaatacctggagaaggggaaggagacgctgcttcacctggagcccccaaagacacacgtgactcaccaccccatctctgaccatgaggccaccctgaggtgctgggccctgggcttctaccctgcggagatcacactgacctggcagcaggatggggagggccatacccaggacacggagctcgtggagaccaggcctgcaggggatggaaccttccagaagtgggcagctgtggtggtgccttctggagaggagcagagatacacgtgccatgtgcagcatgaggggctacccgagcccgtcaccctgagatggaagccggcttcccagcccaccatccccatcgtgggcatcattgctggcctggttctccttggatctgtggtctctggagctgtggttgctgctgtgatatggaggaagaagagctcaggtggaaaaggagggagctactctaaggctgagtggagcgacagtgcccaggggtctgagtctcacagcttg

SEQ ID NO: 27 - DNA, 67 bp, Artificial Sequence
  Synthesized
  misc_feature (3)..(32): n is a, c, g, or t
  misc_feature (43)..(58): n is a, c, g, or t
  misc_feature (63)..(63): n is a, c, g, or t
ctnnnnnnnnnnnnnnnnnnnnnnnnnnnnnncgctccgtggnnnnnnnnnnnnnnnngctanacgt

SEQ ID NO: 28 - DNA, 64 bp, Artificial Sequence
  Synthesized
  misc_feature (3)..(32): n is a, c, g, or t
  misc_feature (45)..(60): n is a, c, g, or t
ctnnnnnnnnnnnnnnnnnnnnnnnnnnnnnncgcgctacttagnnnnnnnnnnnnnnnngcta

SEQ ID NO: 29 - DNA, 63 bp, Artificial Sequence
  Synthesized
  misc_feature (3)..(32): n is a, c, g, or t
  misc_feature (44)..(59): n is a, c, g, or t
ctnnnnnnnnnnnnnnnnnnnnnnnnnnnnnncgcttccgtggnnnnnnnnnnnnnnnngcta

SEQ ID NO: 30 - DNA, 26 bp, Artificial Sequence
  Synthesized
  misc_feature (7)..(22): n is a, c, g, or t
ctaaggnnnnnnnnnnnnnnnngcta

SEQ ID NO: 31 - DNA, 39 bp, Artificial Sequence
  Synthesized
  misc_feature (3)..(32): n is a, c, g, or t
ctnnnnnnnnnnnnnnnnnnnnnnnnnnnnnncgcgcta

SEQ ID NO: 32 - DNA, 61 bp, Artificial Sequence
  Synthesized
  misc_feature (3)..(32): n is a, c, g, or t
  misc_feature (42)..(57): n is a, c, g, or t
ctnnnnnnnnnnnnnnnnnnnnnnnnnnnnnncgcccgtggnnnnnnnnnnnnnnnngcta

SEQ ID NO: 33 - DNA, 7133 bp, Artificial Sequence
  Synthesized
cctgcaggcagctgcgcgctcgctcgctcactgaggccgcccgggcgtcgggcgacctttggtcgcccggcctcagtgagcgagcgagcgcgcagagagggagtggccaactccatcactaggggttcctgcggccgcacgcgtgttctagggtggaaactaagagaatgatgtacctagagggcgctggaagctctaaagccctagcagttactgcttttactattagtggtcgtttttttctcccccccgccccccgacaaatcaacagaacaaagaaaattacctaaacagcaaggacatagggaggaacttcttggcacagaactttccaaacactttttcctgaagggatacaagaagcaagaaaggtactctttcactaggaccttctctgagctgtcctcaggatgcttttgggactatttttcttacccagagaatggagaaaccctgcagggaattcccaagctgtagttataaacagaagttctccttctgctaggtagcattcaaagatcttaatcttctgggtttccgttttctcgaatgaaaaatgcaggtccgagcagttaactggctggggcaccattagcaagtcacttagcatctctggggccagtctgcaaagcgagggggcagccttaatgtgcctccagcctgaagtcctagaatgagcgcccggtgtcccaagctggggcgcgcaccccagatcggagggcgccgatgtacagacagcaaactcacccagtctagtgcatgccttcttaaacatcacgagactctaagaaaaggaaactgaaaacgggaaagtccctctctctaacctggcactgcgtcgctggcttggagacaggtgacggtccctgcgggccttgtcctgattggctgggcacgcgtttaatataagtggaggcgtcgcgctggcgggcattcctgaagctaagcttgtggacgatatcgaattcgcacgacattgattattgactagttattaatagtaatcaattacggggtcattagttcatagcccatatatggagttccgcgttacataacttacggtaaatggcccgcctggctgaccgcccaacgacccccgcccattgacgtcaataatgacgtatgttcccatagtaacgccaatagggactttccattgacgtcaatgggtggactatttacggtaaactgcccacttggcagtacatcaagtgtatcatatgccaagtacgccccctattgacgtcaatgacggtaaatggcccgcctggcattatgcccagtacatgaccttatgggactttcctacttggcagtacatctacgtattagtcatcgctattaccatgggtcgaggtgagccccacgttctgcttcactctccccatctcccccccctccccacccccaattttgtatttatttattttttaattattttgtgcagcgatgggggcggggggggggggggcgcgcgccaggcggggcggggcggggcgaggggcggggcggggcgaggcggagaggtgcggcggcagccaatcagagcggcgcgctccgaaagtttccttttatggcgaggcggcggcggcggcggccctataaaaagcgaagcgcgcggcgggcgggagtcgctgcgttgccttcgccccgtgccccgctccgcgccgcctcgcgccgcccgccccggctctgactgaccgcgttactcccacaggtgagcgggcgggacggcccttctcctccgggctgtaattagcgcttggtttaatgacggctcgtttcttttctgtggctgcgtgaaagccttaaagggctccgggagggccctttgtgcgggggggagcggctcggggggtgcgtgcgtgtgtgtgtgcgtggggagcgccgcgtgcggcccgcgctgcccggcggctgtgagcgctgcgggcgcggcgcggggctttgtgcgctccgcgtgtgcgcgaggggagcgcggccgggggcggtgccccgcggtgcgggggggctgcgaggggaacaaaggctgcgtgcggggtgtgtgcgtgggggggtgagcagggggtgtgggcgcggcggtcgggctgtaacccccccctgcacccccctccccgagttgctgagcacggcccggcttcgggtgcggggctccgtgcggggcgtggcgcggggctcgccgtgccgggcggggggtggcggcaggtgggggtgccgggcggggcggggccgcctcgggccggggagggctcgggggaggggcgcggcggccccggagcgccggcggctgtcgaggcgcggcgagccgcagccattgccttttatggtaatcgtgcgagagggcgcagggacttcctttgtcccaaatctggcggagccgaaatctgggaggcgccgccgcaccccctctagcgggcgcgggcgaagcggtgcggcgccggcaggaaggaaatgggcggggagggccttcgtgcgtcgccgcgccgccgtccccttctccatctccagcctcggggctgccgcagggggacggctgccttcgggggggacggggcagggcggggttcggcttctggcgtgtgaccggcggctctagagcctctgctaaccatgttcatgccttcttctttttcctacaggggggatccgtttatctgcagaattcgcccttgacgtcgccaccatgaggatatttgctgtctttatattcatgacctactggcatttgctgaacgcatttactgtcacggttcccaaggacctatatgtggtagagtatggtagcaatatgacaattgaatgcaaattcccagtagaaaaacaattagacctggctgcactaattgtctattgggaaatggaggataagaacattattcaatttgtgcatggagaggaagacctgaaggttcagcatagtagctacagacagagggcccggctgttgaaggaccagctctccctgggaaatgctgcacttcagatcacagatgtgaaattgcaggatgcaggggtgtaccgctgcatgatcagctatggtggtgccgactacaagcgaattactgtgaaagtcaatgccccatacaacaaaatcaaccaaagaattttggttgtggatccagtcacctctgaacatgaactgacatgtcaggctgagggctaccccaaggccgaagtcatctggacaagcagtgaccatcaagtcctgagtggtaagaccaccaccaccaattccaagagagaggagaaacttttcaatgtgaccagcacactgagaatcaacacaacaactaatgagattttctactgcacttttaggagattagatcctgaggaaaaccatacagctgaattggtcatcccagaactacctctggcacatcctccaaatgaaaggactcacttggtaattctgggagccatcttattatgccttggtgtagcactgacattcatcttccgtttaagaaaagggagaatgatggatgtgaaaaaatgtggcatccaagatacaaactcaaagaagcaaagtgatacacatttggaggagacgtaaccgctgatcagcctcgactgtgccttctagttgccagccatctgttgtttgcccctcccccgtgccttccttgaccctggaaggtgccactcccactgtcctttcctaataaaatgaggaaattgcatcgcattgtctgagtaggtgtcattctattctggggggtggggtggggcaggacagcaagggggaggattgggaagacaatagcaggcatgctggggatgcggtgggctctatgggtcgacccagcgtgagtctctcctaccctcccgctctggtccttcctctcccgctctgcaccctctgtggccctcgctgtgctctctcgctccgtgacttcccttctccaagttctccttggtggcccgccgtggggctagtccagggctggatctcggggaagcggcggggtggcctgggagtggggaagggggtgcgcacccgggacgcgcgctacttgcccctttcggcggggagcaggggagacctttggcctacggcgacgggagggtcgggacaaagtttagggcgtcgataagcgtcagagcgccgaggttgggggagggtttctcttccgctctttcgcggggcctctggctcccccagcgcagctggagtgggggacgggtaggctcgtcccaaaggcgcggcgctgaggtttgtgaacgcgtggaggggcgcttggggtctgggggaggcgtcgcccgggtaagcctgtctgctgcggctctgcttcccttagactggagagctgtggacttcgtctaggcgcccgctaagttcgcatgtcctagcacctctgggtctatgtggggccacaccgtggggaggaaacagcacgcgacgtttgtagaatgcttggctgtgatacaaagcggtttcgaataattaacttatttgttcccatcacatgtcacttttaaaaaattataagaactacccgttattgacatctttctgtgtgccaaggactttatgtgctttgcgtcatttaattttgaaaacagttatcttccgccatagataactactatggttatcttctggtaaccacgtgcggaccgaggctgcagcgtcgtcctccctaggaacccctagtgatggagttggccactccctctctgcgcgctcgctcgctcactgaggccgggcgaccaaaggtcgcccgacgcccgggctttgcccgggcggcctcagtgagcgagcgagcgcgcagctgcctgcaggggcgcctgatgcggtattttctccttacgcatctgtgcggtatttcacaccgcatacgtcaaagcaaccatagtacgcgccctgtagcggcgcattaagcgcggcgggtgtggtggttacgcgcagcgtgaccgctacacttgccagcgccctagcgcccgctcctttcgctttcttcccttcctttctcgccacgttcgccggctttccccgtcaagctctaaatcgggggctccctttagggttccgatttagtgctttacggcacctcgaccccaaaaaacttgatttgggtgatggttcacgtagtgggccatcgccctgatagacggtttttcgccctttgacgttggagtccacgttctttaatagtggactcttgttccaaactggaacaacactcaaccctatctcgggctattcttttgatttataagggattttgccgatttcggcctattggttaaaaaatgagctgatttaacaaaaatttaacgcgaattttaacaaaatattaacgtttacaattttatggtgcactctcagtacaatctgctctgatgccgcatagttaagccagccccgacacccgccaacacccgctgacgcgccctgacgggcttgtctgctcccggcatccgcttacagacaagctgtgaccgtctccgggagctgcatgtgtcagaggttttcaccgtcatcaccgaaacgcgcgagacgaaagggcctcgtgatacgcctatttttataggttaatgtcatgaacaataaaactgtctgcttacataaacagtaatacaaggggtgttatgagccatattcaacgggaaacgtcgaggccgcgattaaattccaacatggatgctgatttatatgggtataaatgggctcgcgataatgtcgggcaatcaggtgcgacaatctatcgcttgtatgggaagcccgatgcgccagagttgtttctgaaacatggcaaaggtagcgttgccaatgatgttacagatgagatggtcagactaaactggctgacggaatttatgcctcttccgaccatcaagcattttatccgtactcctgatgatgcatggttactcaccactgcgatccccggaaaaacagcattccaggtattagaagaatatcctgattcaggtgaaaatattgttgatgcgctggcagtgttcctgcgccggttgcattcgattcctgtttgtaattgtccttttaacagcgatcgcgtatttcgtctcgctcaggcgcaatcacgaatgaataacggtttggttgatgcgagtgattttgatgacgagcgtaatggctggcctgttgaacaagtctggaaagaaatgcataaacttttgccattctcaccggattcagtcgtcactcatggtgatttctcacttgataaccttatttttgacgaggggaaattaataggttgtattgatgttggacgagtcggaatcgcagaccgataccaggatcttgccatcctatggaactgcctcggtgagttttctccttcattacagaaacggctttttcaaaaatatggtattgataatcctgatatgaataaattgcagtttcatttgatgctcgatgagtttttctaatctcatgaccaaaatcccttaacgtgagttttcgttccactgagcgtcagaccccgtagaaaagatcaaaggatcttcttgagatcctttttttctgcgcgtaatctgctgcttgcaaacaaaaaaaccaccgctaccagcggtggtttgtttgccggatcaagagctaccaactctttttccgaaggtaactggcttcagcagagcgcagataccaaatactgtccttctagtgtagccgtagttaggccaccacttcaagaactctgtagcaccgcctacatacctcgctctgctaatcctgttaccagtggctgctgccagtggcgataagtcgtgtcttaccgggttggactcaagacgatagttaccggataaggcgcagcggtcgggctgaacggggggttcgtgcacacagcccagcttggagcgaacgacctacaccgaactgagatacctacagcgtgagctatgagaaagcgccacgcttcccgaagggagaaaggcggacaggtatccggtaagcggcagggtcggaacaggagagcgcacgagggagcttccagggggaaacgcctggtatctttatagtcctgtcgggtttcgccacctctgacttgagcgtcgatttttgtgatgctcgtcaggggggcggagcctatggaaaaacgccagcaacgcggcctttttacggttcctggccttttgctggccttttgctcacatgt

SEQ ID NO: 34 - DNA, 7763 bp, Artificial Sequence
  Synthesized
cctgcaggcagctgcgcgctcgctcgctcactgaggccgcccgggcgtcgggcgacctttggtcgcccggcctcagtgagcgagcgagcgcgcagagagggagtggccaactccatcactaggggttcctgcggccgcacgcgtgttctagggtggaaactaagagaatgatgtacctagagggcgctggaagctctaaagccctagcagttactgcttttactattagtggtcgtttttttctcccccccgccccccgacaaatcaacagaacaaagaaaattacctaaacagcaaggacatagggaggaacttcttggcacagaactttccaaacactttttcctgaagggatacaagaagcaagaaaggtactctttcactaggaccttctctgagctgtcctcaggatgcttttgggactatttttcttacccagagaatggagaaaccctgcagggaattcccaagctgtagttataaacagaagttctccttctgctaggtagcattcaaagatcttaatcttctgggtttccgttttctcgaatgaaaaatgcaggtccgagcagttaactggctggggcaccattagcaagtcacttagcatctctggggccagtctgcaaagcgagggggcagccttaatgtgcctccagcctgaagtcctagaatgagcgcccggtgtcccaagctggggcgcgcaccccagatcggagggcgccgatgtacagacagcaaactcacccagtctagtgcatgccttcttaaacatcacgagactctaagaaaaggaaactgaaaacgggaaagtccctctctctaacctggcactgcgtcgctggcttggagacaggtgacggtccctgcgggccttgtcctgattggctgggcacgcgtttaatataagtggaggcgtcgcgctggcgggcattcctgaagctaagcttgtggacgatatcgaattcgcacgacattgattattgactagttattaatagtaatcaattacggggtcattagttcatagcccatatatggagttccgcgttacataacttacggtaaatggcccgcctggctgaccgcccaacgacccccgcccattgacgtcaataatgacgtatgttcccatagtaacgccaatagggactttccattgacgtcaatgggtggactatttacggtaaactgcccacttggcagtacatcaagtgtatcatatgccaagtacgccccctattgacgtcaatgacggtaaatggcccgcctggcattatgcccagtacatgaccttatgggactttcctacttggcagtacatctacgtattagtcatcgctattaccatgggtcgaggtgagccccacgttctgcttcactctccccatctcccccccctccccacccccaattttgtatttatttattttttaattattttgtgcagcgatgggggcggggggggggggggcgcgcgccaggcggggcggggcggggcgaggggcggggcggggcgaggcggagaggtgcggcggcagccaatcagagcggcgcgctccgaaagtttccttttatggcgaggcggcggcggcggcggccctataaaaagcgaagcgcgcggcgggcgggagtcgctgcgttgccttcgccccgtgccccgctccgcgccgcctcgcgccgcccgccccggctctgactgaccgcgttactcccacaggtgagcgggcgggacggcccttctcctccgggctgtaattagcgcttggtttaatgacggctcgtttcttttctgtggctgcgtgaaagccttaaagggctccgggagggccctttgtgcgggggggagcggctcggggggtgcgtgcgtgtgtgtgtgcgtggggagcgccgcgtgcggcccgcgctgcccggcggctgtgagcgctgcgggcgcggcgcggggctttgtgcgctccgcgtgtgcgcgaggggagcgcggccgggggcggtgccccgcggtgcgggggggctgcgaggggaacaaaggctgcgtgcggggtgtgtgcgtgggggggtgagcagggggtgtgggcgcggcggtcgggctgtaacccccccctgcacccccctccccgagttgctgagcacggcccggcttcgggtgcggggctccgtgcggggcgtggcgcggggctcgccgtgccgggcggggggtggcggcaggtgggggtgccgggcggggcggggccgcctcgggccggggagggctcgggggaggggcgcggcggccccggagcgccggcggctgtcgaggcgcggcgagccgcagccattgccttttatggtaatcgtgcgagagggcgcagggacttcctttgtcccaaatctggcggagccgaaatctgggaggcgccgccgcaccccctctagcgggcgcgggcgaagcggtgcggcgccggcaggaaggaaatgggcggggagggccttcgtgcgtcgccgcgccgccgtccccttctccatctccagcctcggggctgccgcagggggacggctgccttcgggggggacggggcagggcggggttcggcttctggcgtgtgaccggcggctctagagcctctgctaaccatgttcatgccttcttctttttcctacaggggggatccgtttatctgcagaattcgcccttgacgtcgccaccatgtctcgctccgtggccttagctgtgctcgcgctactctctctttctggcctggaggctgtcatggcgccccgaaccctcttcctgggtggaggcggttcaggcggaggtggctctggcggtggcggatcgatccagcgtactccaaagattcaggtttactcacgtcatccagcagagaatggaaagtcaaatttcctgaattgctatgtgtctgggtttcatccatccgacattgaagttgacttactgaagaatggagagagaattgaaaaagtggagcattcagacttgtctttcagcaaggactggtctttctatctcttgtactacactgaattcacccccactgaaaaagatgagtatgcctgccgtgtgaaccatgtgactttgtcacagcccaagatagttaagtgggatcgagacatgggtggtggtggttctggtggtggtggttctggcggcggcggctccggtggtggtggatccggctcccactccttgaagtatttccacacttccgtgtcccggcccggccgcggggagccccgcttcatctctgtgggctacgtggacgacacccagttcgtgcgcttcgacaacgacgccgcgagtccgaggatggtgccgcgggcgccgtggatggagcaggaggggtcagagtattgggaccgggagacacggagcgccagggacaccgcacagattttccgagtgaatctgcggacgctgcgcggctactacaatcagagcgaggccgggtctcacaccctgcagtggatgcatggctgcgagctggggcccgacgggcgcttcctccgcgggtatgaacagttcgcctacgacggcaaggattatctcaccctgaatgaggacctgcgctcctggaccgcggtggacacggcggctcagatctccgagcaaaagtcaaatgatgcctctgaggcggagcaccagagagcctacctggaagacacatgcgtggagtggctccacaaatacctggagaaggggaaggagacgctgcttcacctggagcccccaaagacacacgtgactcaccaccccatctctgaccatgaggccaccctgaggtgctgggccctgggcttctaccctgcggagatcacactgacctggcagcaggatggggagggccatacccaggacacggagctcgtggagaccaggcctgcaggggatggaaccttccagaagtgggcagctgtggtggtgccttctggagaggagcagagatacacgtgccatgtgcagcatgaggggctacccgagcccgtcaccctgagatggaagccggcttcccagcccaccatccccatcgtgggcatcattgctggcctggttctccttggatctgtggtctctggagctgtggttgctgctgtgatatggaggaagaagagctcaggtggaaaaggagggagctactctaaggctgagtggagcgacagtgcccaggggtctgagtctcacagcttgtaaccgctgatcagcctcgactgtgccttctagttgccagccatctgttgtttgcccctcccccgtgccttccttgaccctggaaggtgccactcccactgtcctttcctaataaaatgaggaaattgcatcgcattgtctgagtaggtgtcattctattctggggggtggggtggggcaggacagcaagggggaggattgggaagacaatagcaggcatgctggggatgcggtgggctctatgggtcgacccagcgtgagtctctcctaccctcccgctctggtccttcctctcccgctctgcaccctctgtggccctcgctgtgctctctcgctccgtgacttcccttctccaagttctccttggtggcccgccgtggggctagtccagggctggatctcggggaagcggcggggtggcctgggagtggggaagggggtgcgcacccgggacgcgcgctacttgcccctttcggcggggagcaggggagacctttggcctacggcgacgggagggtcgggacaaagtttagggcgtcgataagcgtcagagcgccgaggttgggggagggtttctcttccgctctttcgcggggcctctggctcccccagcgcagctggagtgggggacgggtaggctcgtcccaaaggcgcggcgctgaggtttgtgaacgcgtggaggggcgcttggggtctgggggaggcgtcgcccgggtaagcctgtctgctgcggctctgcttcccttagactggagagctgtggacttcgtctaggcgcccgctaagttcgcatgtcctagcacctctgggtctatgtggggccacaccgtggggaggaaacagcacgcgacgtttgtagaatgcttggctgtgatacaaagcggtttcgaataattaacttatttgttcccatcacatgtcacttttaaaaaattataagaactacccgttattgacatctttctgtgtgccaaggactttatgtgctttgcgtcatttaattttgaaaacagttatcttccgccatagataactactatggttatcttctggtaaccacgtgcggaccgaggctgcagcgtcgtcctccctaggaacccctagtgatggagttggccactccctctctgcgcgctcgctcgctcactgaggccgggcgaccaaaggtcgcccgacgcccgggctttgcccgggcggcctcagtgagcgagcgagcgcgcagctgcctgcaggggcgcctgatgcggtattttctccttacgcatctgtgcggtatttcacaccgcatacgtcaaagcaaccatagtacgcgccctgtagcggcgcattaagcgcggcgggtgtggtggttacgcgcagcgtgaccgctacacttgccagcgccctagcgcccgctcctttcgctttcttcccttcctttctcgccacgttcgccggctttccccgtcaagctctaaatcgggggctccctttagggttccgatttagtgctttacggcacctcgaccccaaaaaacttgatttgggtgatggttcacgtagtgggccatcgccctgatagacggtttttcgccctttgacgttggagtccacgttctttaatagtggactcttgttccaaactggaacaacactcaaccctatctcgggctattcttttgatttataagggattttgccgatttcggcctattggttaaaaaatgagctgatttaacaaaaatttaacgcgaattttaacaaaatattaacgtttacaattttatggtgcactctcagtacaatctgctctgatgccgcatagttaagccagccccgacacccgccaacacccgctgacgcgccctgacgggcttgtctgctcccggcatccgcttacagacaagctgtgaccgtctccgggagctgcatgtgtcagaggttttcaccgtcatcaccgaaacgcgcgagacgaaagggcctcgtgatacgcctatttttataggttaatgtcatgaacaataaaactgtctgcttacataaacagtaatacaaggggtgttatgagccatattcaacgggaaacgtcgaggccgcgattaaattccaacatggatgctgatttatatgggtataaatgggctcgcgataatgtcgggcaatcaggtgcgacaatctatcgcttgtatgggaagcccgatgcgccagagttgtttctgaaacatggcaaaggtagcgttgccaatgatgttacagatgagatggtcagactaaactggctgacggaatttatgcctcttccgaccatcaagcattttatccgtactcctgatgatgcatggttactcaccactgcgatccccggaaaaacagcattccaggtattagaagaatatcctgattcaggtgaaaatattgttgatgcgctggcagtgttcctgcgccggttgcattcgattcctgtttgtaattgtccttttaacagcgatcgcgtatttcgtctcgctcaggcgcaatcacgaatgaataacggtttggttgatgcgagtgattttgatgacgagcgtaatggctggcctgttgaacaagtctggaaagaaatgcataaacttttgccattctcaccggattcagtcgtcactcatggtgatttctcacttgataaccttatttttgacgaggggaaattaataggttgtattgatgttggacgagtcggaatcgcagaccgataccaggatcttgccatcctatggaactgcctcggtgagttttctccttcattacagaaacggctttttcaaaaatatggtattgataatcctgatatgaataaattgcagtttcatttgatgctcgatgagtttttctaatctcatgaccaaaatcccttaacgtgagttttcgttccactgagcgtcagaccccgtagaaaagatcaaaggatcttcttgagatcctttttttctgcgcgtaatctgctgcttgcaaacaaaaaaaccaccgctaccagcggtggtttgtttgccggatcaagagctaccaactctttttccgaaggtaactggcttcagcagagcgcagataccaaatactgtccttctagtgtagccgtagttaggccaccacttcaagaactctgtagcaccgcctacatacctcgctctgctaatcctgttaccagtggctgctgccagtggcgataagtcgtgtcttaccgggttggactcaagacgatagttaccggataaggcgcagcggtcgggctgaacggggggttcgtgcacacagcccagcttggagcgaacgacctacaccgaactgagatacctacagcgtgagctatgagaaagcgccacgcttcccgaagggagaaaggcggacaggtatccggtaagcggcagggtcggaacaggagagcgcacgagggagcttccagggggaaacgcctggtatctttatagtcctgtcgggtttcgccacctctgacttgagcgtcgatttttgtgatgctcgtcaggggggcggagcctatggaaaaacgccagcaacgcggcctttttacggttcctggccttttgctggccttttgctcacatgt

SEQ ID NO: 35 - DNA, 20 bp, Homo sapiens
tataagtggaggcgtcgcgc

SEQ ID NO: 36 - DNA, 20 bp, Homo sapiens
gagtagcgcgagcacagcta

SEQ ID NO: 37 - DNA, 20 bp, Homo sapiens
actggacgcgtcgcgctggc

SEQ ID NO: 38 - DNA, 20 bp, Homo sapiens
aagtggaggcgtcgcgctgg

SEQ ID NO: 39 - DNA, 20 bp, Homo sapiens
ggccacggagcgagacatct

SEQ ID NO: 40 - DNA, 20 bp, Homo sapiens
gcccgaatgctgtcagcttc

SEQ ID NO: 41 - DNA, 20 bp, Homo sapiens
ctcgcgctactctctctttc

SEQ ID NO: 42 - DNA, 20 bp, Homo sapiens
tcctgaagctgacagcattc

SEQ ID NO: 43 - DNA, 20 bp, Homo sapiens
ttcctgaagctgacagcatt

SEQ ID NO: 44 - DNA, 20 bp, Homo sapiens
actctctctttctggcctgg